European Patent Application EP 4 428 148 A1, published September 11, 2024. Title: RECOMBINANT COLLAGEN AND PREPARATION METHOD AND USE THEREOF. Applicant: JIANGSU TRAUTEC MEDICAL TECHNOLOGY CO., LTD. The sequence listing filed with the application follows.

SEQUENCE LISTING (10 sequences)

SEQ ID NO: 1 - protein, 1057 aa, Homo sapiens
QLSYGYDEKSTGGISVPGPMGPSGPRGLPGPPGAPGPQGFQGPPGEPGEPGASGPMGPRGPPGPPGKNGDDGEAGKPGRPGERGPPGPQGARGLPGTAGLPGMKGHRGFSGLDGAKGDAGPAGPKGEPGSPGENGAPGQMGPRGLPGERGRPGAPGPAGARGNDGATGAAGPPGPTGPAGPPGFPGAVGAKGEAGPQGPRGSEGPQGVRGEPGPPGPAGAAGPAGNPGADGQPGAKGANGAPGIAGAPGFPGARGPSGPQGPGGPPGPKGNSGEPGAPGSKGDTGAKGEPGPVGVQGPPGPAGEEGKRGARGEPGPTGLPGPPGERGGPGSRGFPGADGVAGPKGPAGERGSPGPAGPKGSPGEAGRPGEAGLPGAKGLTGSPGSPGPDGKTGPPGPAGQDGRPGPPGPPGARGQAGVMGFPGPKGAAGEPGKAGERGVPGPPGAVGPAGKDGEAGAQGPPGPAGPAGERGEQGPAGSPGFQGLPGPAGPPGEAGKPGEQGVPGDLGAPGPSGARGERGFPGERGVQGPPGPAGPRGANGAPGNDGAKGDAGAPGAPGSQGAPGLQGMPGERGAAGLPGPKGDRGDAGPKGADGSPGKDGVRGLTGPIGPPGPAGAPGDKGESGPSGPAGPTGARGAPGDRGEPGPPGPAGFAGPPGADGQPGAKGEPGDAGAKGDAGPPGPAGPAGPPGPIGNVGAPGAKGARGSAGPPGATGFPGAAGRVGPPGPSGNAGPPGPPGPAGKEGGKGPRGETGPAGRPGEVGPPGPPGPAGEKGSPGADGPAGAPGTPGPQGIAGQRGVVGLPGQRGERGFPGLPGPSGEPGKQGPSGASGERGPPGPMGPPGLAGPPGESGREGAPGAEGSPGRDGSPGAKGDRGETGPAGPPGAPGAPGAPGPVGPAGKSGDRGETGPAGPAGPVGPVGARGPAGPQGPRGDKGETGEQGDRGIKGHRGFSGLQGPPGPPGSPGEQGPSGASGPAGPRGPPGSAGAPGKDGLNGLPGPIGPPGPRGRTGDAGPVGPPGPPGPPGPPGPPSAGFDFSFLPQPPQEKAHDGGRYYRA

SEQ ID NO: 2 - protein, 1057 aa, Artificial Sequence
  source 1..1057: note = Amino acid sequence of a1 (I) M1
QLSYGYDEKSTGGISVPGPMGPSGPRGLPGPPGAPGPQGFQGPPGEPGEPGASGPPGPPGPPGPPGKNGDDGEAGKPGRPGERGPPGPQGARGLPGTAGLPGMKGHRGFSGLDGAKGDAGPAGPKGEPGSPGENGAPGQPGPPGLPGERGRPGAPGPAGARGNDGATGAAGPPGPTGPAGPPGFPGAVGAKGEAGPQGPRGSEGPQGVRGEPGPPGPAGAAGPAGNPGADGQPGAKGANGAPGIAGAPGFPGARGPSGPQGPGGPPGPKGNSGEPGAPGSKGDTGAKGEPGPVGVQGPPGPAGEEGKRGARGEPGPTGLPGPPGERGGPGSRGFPGADGVAGPKGPAGERGSPGPAGPKGSPGEAGRPGEAGLPGAKGLTGSPGSPGPDGKTGPPGPAGQDGRPGPPGPPGARGQAGVMGFPGPKGAAGEPGKAGERGVPGPPGAVGPAGKDGEAGAQGPPGPAGPAGERGEQGPAGSPGFQGLPGPAGPPGEAGKPGEQGVPGDLGAPGPSGARGERGFPGERGVQGPPGPAGPRGANGAPGNDGAKGDAGAPGAPGSQGAPGLQGMPGERGAAGLPGPKGDRGDAGPKGADGSPGKDGVRGLTGPIGPPGPAGAPGDKGESGPSGPAGPTGARGAPGDRGEPGPPGPAGFAGPPGADGQPGAKGEPGDAGAKGDAGPPGPAGPAGPPGPIGNVGAPGAKGARGSAGPPGATGFPGAAGRVGPPGPSGNAGPPGPPGPAGKEGGKGPRGETGPAGRPGEVGPPGPPGPAGEKGSPGADGPAGAPGTPGPQGIAGQRGVVGLPGQRGERGFPGLPGPSGEPGKQGPSGASGERGPPGPMGPPGLAGPPGESGREGAPGAEGSPGRDGSPGAKGDRGETGPAGPPGAPGAPGAPGPVGPAGKSGDRGETGPAGPAGPVGPVGARGPAGPQGPRGDKGETGEQGDRGIKGHRGFSGLQGPPGPPGSPGEQGPSGASGPAGPRGPPGSAGAPGKDGLNGLPGPIGPPGPRGRTGDAGPVGPPGPPGPPGPPGPPSAGFDFSFLPQPPQEKAHDGGRYYRA

SEQ ID NO: 3 - DNA, 3171 bp, Artificial Sequence
  source 1..3171: mol_type = other DNA; note = Nucleotide sequence encoding a1 (I) M1
caacttagttatggatacgatgaaaaatccacaggtggaatcagtgttcctggacctatgggtccatcaggtccaagaggtttaccaggacctccaggtgccccaggtccccagggatttcaaggtccaccaggagagcctggtgagccaggagcttctggtccacctggtccccctggaccacctggtcctccaggaaagaatggagatgatggtgaagctggaaaacctggaagacctggagaaagaggaccaccaggaccccagggtgccagaggactgccaggtaccgcaggtctgcctggaatgaaaggtcatagaggattttcaggattagacggtgcaaagggagacgctggacctgcaggaccaaagggtgagccaggaagtccaggagagaatggtgcaccaggacagccaggtccacctggactgcccggtgaaagaggtagacccggagcaccaggaccagcaggtgcaagaggaaatgatggagctacaggtgctgcaggacccccaggtccaacaggaccagccggtcctcccggtttcccaggtgccgttggagcaaaaggtgaagctggtccacagggtccaagaggttctgaaggtccacagggagttagaggagaaccaggaccccctggaccagctggtgcagcaggaccagctggtaaccctggtgctgacggtcagccaggtgctaagggagcaaatggagcaccaggaatagctggtgccccaggatttcccggtgctagaggtccaagtggtccacaaggaccaggaggtccacccggtcccaaaggaaacagtggagaaccaggtgcacccggttcaaagggagatacaggagctaaaggagagcccggtccagtgggtgttcagggaccacccggacctgctggagaggaaggtaaaagaggtgcaagaggtgagccaggaccaacaggtctgcctggtccccctggtgaaagaggtggtccaggtagtagaggatttccaggagctgatggtgttgcaggaccaaagggacccgcaggtgagagaggatcacccggtccagccggaccaaaaggatcaccaggagaagctggtagaccaggagaagctggtctgccaggtgctaaaggattgacaggatcacccggttcacctggtcctgatggaaagacaggacctccaggtcccgctggtcaggacggtagaccaggacccccaggacccccaggtgcaagaggtcaggcaggtgtaatgggtttccccggacctaaaggagcagctggagaacctggtaaagctggagagagaggagtgcctggaccccctggagctgttggtccagcaggaaaggatggtgaggcaggtgcacaaggtccacctggacccgctggacctgcaggtgagagaggagagcaaggtcccgcaggttctccaggttttcagggtttgccaggtccagccggtcctcctggagaggcaggaaagccaggagaacaaggagttccaggagacctgggtgcaccaggaccctctggtgcaagaggagagagaggatttcctggagaaagaggtgtgcagggaccaccaggtcccgccggtccaagaggagcaaatggagcccctggaaatgacggagctaagggtgacgctggtgcaccaggagcaccaggttctcaaggtgctcccggattgcagggtatgcctggagagagaggtgcagctggactgccaggtccaaaaggtgacagaggagacgccggtcctaagggagctgacggttctcctggaaaggacggtgtgagaggtttgacaggaccaataggtccacccggtcctgctggagcccctggagacaaaggtgaatcaggtccttccggtccagccggaccaacaggagcaagaggagcacctggagacagaggagagccaggtcctccaggacctgcaggtttcgctggtcctcccggagcagatggacagccaggagctaagggagaacccggtgacgctggtgctaagggagatgcaggtccaccaggtcctgctggtcctgctggacctcccggaccaataggtaatgttggagcacccggagcaaaaggtgccagaggttccgcaggtcctcccggagcaactggttttccaggagctgccggaagagtgggtccacctggtccttctggaaatgcaggaccaccaggtcctcctggtccagccggaaaggaaggtggaaagggacctagaggagaaacaggtcccgcaggtagacccggtgaggtgggtccacctggtccacccggtccagctggtgagaaaggaagtcctggagcagacggaccagctggtgcccctggtacaccaggaccccaaggaatagctggtcaaagaggtgttgttggtttaccaggtcagagaggagaaagaggttttccaggattaccaggtccctcaggtgagcccggaaaacagggtccctcaggagcaagtggtgaaagaggaccaccaggaccaatgggacctccaggattagctggtccaccaggagaatcaggaagagagggtgctcctggagcagaaggttcaccaggaagagacggttcacccggagccaagggagacagaggtgaaacaggtcccgcaggtccaccaggagcacccggagcccctggtgctccaggacctgtcggaccagcaggaaaatccggtgacagaggtgagactggacccgcaggtcctgctggtcctgttggaccagtgggtgcaagaggaccagcaggtccacaaggtccaagaggtgacaaaggtgagacaggtgagcagggtgacagaggaattaaaggtcacagaggattttcaggactgcagggaccacccggtcctcccggttccccaggagagcaaggtccatccggtgcatccggtccagctggacccagaggaccacctggttctgctggtgcaccaggtaaagatggattgaacggtttgcctggtccaataggacctcctggtccaagaggaagaactggtgacgccggtcccgtcggaccacccggtccaccaggtcccccaggtccacccggaccaccatccgcaggatttgatttctcattccttcctcaacctcctcaagagaaagcacatgatggaggtagatactatagagcc

SEQ ID NO: 4 - protein, 1060 aa, Homo sapiens
QMAGGFDEKAGGAQLGVMQGPMGPMGPRGPPGPAGAPGPQGFQGNPGEPGEPGVSGPMGPRGPPGPPGKPGDDGEAGKPGKAGERGPPGPQGARGFPGTPGLPGVKGHRGYPGLDGAKGEAGAPGVKGESGSPGENGSPGPMGPRGLPGERGRTGPAGAAGARGNDGQPGPAGPPGPVGPAGGPGFPGAPGAKGEAGPTGARGPEGAQGPRGEPGTPGSPGPAGASGNPGTDGIPGAKGSAGAPGIAGAPGFPGPRGPPGPQGATGPLGPKGQTGEPGIAGFKGEQGPKGEPGPAGPQGAPGPAGEEGKRGARGEPGGVGPIGPPGERGAPGNRGFPGQDGLAGPKGAPGERGPSGLAGPKGANGDPGRPGEPGLPGARGLTGRPGDAGPQGKVGPSGAPGEDGRPGPPGPQGARGQPGVMGFPGPKGANGEPGKAGEKGLPGAPGLRGLPGKDGETGAAGPPGPAGPAGERGEQGAPGPSGFQGLPGPPGPPGEGGKPGDQGVPGEAGAPGLVGPRGERGFPGERGSPGAQGLQGPRGLPGTPGTDGPKGASGPAGPPGAQGPPGLQGMPGERGAAGIAGPKGDRGDVGEKGPEGAPGKDGGRGLTGPIGPPGPAGANGEKGEVGPPGPAGSAGARGAPGERGETGPPGPAGFAGPPGADGQPGAKGEQGEAGQKGDAGAPGPQGPSGAPGPQGPTGVTGPKGARGAQGPPGATGFPGAAGRVGPPGSNGNPGPPGPPGPSGKDGPKGARGDSGPPGRAGEPGLQGPAGPPGEKGEPGDDGPSGAEGPPGPQGLAGQRGIVGLPGQRGERGFPGLPGPSGEPGKQGAPGASGDRGPPGPVGPPGLTGPAGEPGREGSPGADGPPGRDGAAGVKGDRGETGAVGAPGAPGPPGSPGPAGPTGKQGDRGEAGAQGPMGPSGPAGARGIQGPQGPRGDKGEAGEPGERGLKGHRGFTGLQGLPGPPGPSGDQGASGPAGPSGPRGPPGPVGPSGKDGANGIPGPIGPPGPRGRSGETGPAGPPGNPGPPGPPGPPGPGIDMSAFAGLGPREKGPDPLQYMRA

SEQ ID NO: 5 - protein, 1060 aa, Artificial Sequence
  source 1..1060: note = Amino acid sequence of a1 (II) M6
QMAGGFDEKAGGAQLGPPQGPPGPPGPPGPPGPAGAPGPQGFQGNPGEPGEPGVSGPPGPPGPPGPPGKPGDDGEAGKPGKAGERGPPGPQGARGFPGTPGLPGVKGHRGYPGLDGAKGEAGAPGVKGESGSPGENGSPGPPGPPGLPGERGRTGPAGAAGARGNDGQPGPAGPPGPVGPAGGPGFPGAPGAKGEAGPTGARGPEGAQGPRGEPGTPGSPGPAGASGNPGTDGIPGAKGSAGAPGIAGAPGFPGPRGPPGPQGATGPLGPKGQTGEPGIAGFKGEQGPKGEPGPAGPQGAPGPAGEEGKRGARGEPGGVGPIGPPGERGAPGNRGFPGQDGLAGPKGAPGERGPSGLAGPKGANGDPGRPGEPGLPGARGLTGRPGDAGPQGKVGPSGAPGEDGRPGPPGPQGARGQPGVMGFPGPKGANGEPGKAGEKGLPGAPGLRGLPGKDGETGAAGPPGPAGPAGERGEQGAPGPSGFQGLPGPPGPPGEGGKPGDQGVPGEAGAPGLVGPRGERGFPGERGSPGAQGLQGPRGLPGTPGTDGPKGASGPAGPPGAQGPPGLQGMPGERGAAGIAGPKGDRGDVGEKGPEGAPGKDGGRGLTGPIGPPGPAGANGEKGEVGPPGPAGSAGARGAPGERGETGPPGPAGFAGPPGADGQPGAKGEQGEAGQKGDAGAPGPQGPSGAPGPQGPTGVTGPKGARGAQGPPGATGFPGAAGRVGPPGSNGNPGPPGPPGPSGKDGPKGARGDSGPPGRAGEPGLQGPAGPPGEKGEPGDDGPSGAEGPPGPQGLAGQRGIVGLPGQRGERGFPGLPGPSGEPGKQGAPGASGDRGPPGPVGPPGLTGPAGEPGREGSPGADGPPGRDGAAGVKGDRGETGAVGAPGAPGPPGSPGPAGPTGKQGDRGEAGAQGPMGPSGPAGARGIQGPQGPRGDKGEAGEPGERGLKGHRGFTGLQGLPGPPGPSGDQGASGPAGPSGPRGPPGPVGPSGKDGANGIPGPIGPPGPRGRSGETGPAGPPGNPGPPGPPGPPGPGIDMSAFAGLGPREKGPDPLQYMRA

SEQ ID NO: 6 - DNA, 3180 bp, Artificial Sequence
  source 1..3180: mol_type = other DNA; note = Nucleotide sequence encoding a1 (II) M6
caaatggctggtggattcgatgaaaaggctggtggagcccaattaggtcctccacaaggtcctcccggtccacctggtcctcccggtcctccaggtcccgccggtgctcctggaccacagggtttccaaggaaaccccggtgaaccaggtgagcctggtgtttcaggtcctcccggtcctccaggaccacctggaccaccaggaaagcctggtgacgacggagaagctggtaaaccaggaaaggcaggagagagaggtccacctggacctcagggtgccagaggtttcccaggtacccctggtcttcctggtgtcaagggtcatagaggttaccccggtttggatggtgccaagggtgaagccggtgcccctggtgttaagggtgaatcaggaagtcccggtgaaaatggaagtcccggtccacccggtccacctggactgccaggtgagagaggaagaaccggaccagctggtgctgcaggtgctagaggaaatgacggacagcccggaccagccggacctcccggtcctgttgggcccgcaggtggtcctggtttccctggtgctcctggagccaaaggagaagccggacccaccggagccagaggtcccgagggagcacagggacctagaggagaaccaggtacaccaggtagtcccggtcctgctggtgcatcaggaaatcccggaactgacggtattccaggagcaaagggatctgcaggagcaccaggaatagctggtgctcctggatttccaggtcccagaggacctcccggtcctcaaggagcaacaggtcctttgggaccaaaaggtcaaacaggagaaccaggtattgctggattcaaaggagagcaaggtccaaagggagagcccggtcccgcaggtccccaaggagccccaggaccagctggtgaagaaggaaaaagaggagccagaggtgaacctggaggagtaggacctattggtcctcctggtgagagaggtgctcccggaaacagaggttttcctggtcaagatggtctggctggacctaaaggtgctccaggagagagaggaccttcaggacttgctggtccaaaaggtgctaacggagatccaggaagacccggtgaacctggtctgcctggagctagaggattaacaggaagaccaggtgacgcaggtccccagggtaaagtgggtcccagtggtgccccaggtgaagatggaagacctggtcctcccggaccccaaggtgcaagaggtcagcctggagtgatgggatttcctggacccaagggtgctaacggagaacctggaaaagctggtgagaaaggactgcccggtgccccaggtcttagaggtttgccaggtaaagatggagaaacaggagccgcaggaccacccggtccagccggaccagcaggagagagaggtgaacaaggagcacctggtccaagtggttttcagggtcttccaggtccccctggtccaccaggagagggaggtaaaccaggtgaccaaggtgtccctggagaagcaggtgcacccggtcttgtgggtccaagaggtgaaagaggattccctggtgagagaggatctcccggagcccagggacttcaaggtcctagaggtctgccaggtacccctggtacagacggaccaaagggagcatcaggacccgctggacctcccggagcccaaggtcctccaggtttacaaggtatgcctggtgaaagaggtgctgcaggtatagctggaccaaaaggagacagaggtgacgttggtgagaagggtcccgaaggagcccctggaaaagatggtggaagaggattaacaggtcctataggaccacccggtccagccggtgctaatggagaaaaaggagaagtaggtcctccaggtccagcaggatctgcaggtgctagaggtgcccctggagagagaggtgaaacaggaccacctggtccagctggtttcgctggtcccccaggagctgatggacagcccggtgcaaaaggtgaacaaggagaagccggacagaagggagatgctggagcccccggtccacaaggtccctcaggagcaccaggtcctcaaggtccaactggtgtgaccgggccaaagggtgcaagaggagcacagggacctccaggagcaacaggtttcccaggagctgctggtagagtcggtccacccggatctaatggtaaccccggaccaccaggaccacctggaccatctggaaaggatggacccaaaggagcaagaggagattcaggaccacccggaagagcaggagaacctggattacagggtcccgccggtccaccaggagagaaaggagagcccggagatgatggtccctcaggtgcagagggacccccaggaccccaaggtctggcaggtcaaagaggtatagtgggtcttccaggtcaaagaggtgaaagaggatttccaggacttccaggtccttcaggtgaacccggtaaacagggagcccccggagcctcaggtgacagaggtcctccaggaccagtaggacccccaggtttaaccggaccagcaggtgagccaggaagagaaggttctcctggagccgatggacctccaggaagagacggtgcagctggtgttaagggtgacagaggtgaaactggagccgtaggagccccaggtgcccccggaccacccggatcacccggacctgcaggtcctactggtaaacaaggagatagaggagaagccggtgcccagggtcctatgggtccttctggtcctgcaggagcaagaggtatacaaggtccacagggtcccagaggtgacaagggtgaagcaggagaacccggtgagagaggtctgaagggtcatagaggattcaccgggttacagggtttgccaggaccccctggaccaagtggtgaccagggtgcatccggtccagcaggtccttctggaccaagaggtcctcccggtccagttggtccatcaggtaaagacggagccaacggtatcccaggtcccatcggtcctccaggtcctagaggaagaagtggagagactggtcctgctggacctcctggaaaccctggtcctccaggacctccaggtcctccaggtcccggaatagatatgtccgctttcgctggattgggaccaagagagaaaggtcctgaccctcttcaatatatgagagca

SEQ ID NO: 7 - protein, 1071 aa, Artificial Sequence
  source 1..1071: note = Amino acid sequence of a1 (I) M1 with N-terminal Strep-Tag II tag and C-terminal 6 x His Tag
WSHPQFEKQLSYGYDEKSTGGISVPGPMGPSGPRGLPGPPGAPGPQGFQGPPGEPGEPGASGPPGPPGPPGPPGKNGDDGEAGKPGRPGERGPPGPQGARGLPGTAGLPGMKGHRGFSGLDGAKGDAGPAGPKGEPGSPGENGAPGQPGPPGLPGERGRPGAPGPAGARGNDGATGAAGPPGPTGPAGPPGFPGAVGAKGEAGPQGPRGSEGPQGVRGEPGPPGPAGAAGPAGNPGADGQPGAKGANGAPGIAGAPGFPGARGPSGPQGPGGPPGPKGNSGEPGAPGSKGDTGAKGEPGPVGVQGPPGPAGEEGKRGARGEPGPTGLPGPPGERGGPGSRGFPGADGVAGPKGPAGERGSPGPAGPKGSPGEAGRPGEAGLPGAKGLTGSPGSPGPDGKTGPPGPAGQDGRPGPPGPPGARGQAGVMGFPGPKGAAGEPGKAGERGVPGPPGAVGPAGKDGEAGAQGPPGPAGPAGERGEQGPAGSPGFQGLPGPAGPPGEAGKPGEQGVPGDLGAPGPSGARGERGFPGERGVQGPPGPAGPRGANGAPGNDGAKGDAGAPGAPGSQGAPGLQGMPGERGAAGLPGPKGDRGDAGPKGADGSPGKDGVRGLTGPIGPPGPAGAPGDKGESGPSGPAGPTGARGAPGDRGEPGPPGPAGFAGPPGADGQPGAKGEPGDAGAKGDAGPPGPAGPAGPPGPIGNVGAPGAKGARGSAGPPGATGFPGAAGRVGPPGPSGNAGPPGPPGPAGKEGGKGPRGETGPAGRPGEVGPPGPPGPAGEKGSPGADGPAGAPGTPGPQGIAGQRGVVGLPGQRGERGFPGLPGPSGEPGKQGPSGASGERGPPGPMGPPGLAGPPGESGREGAPGAEGSPGRDGSPGAKGDRGETGPAGPPGAPGAPGAPGPVGPAGKSGDRGETGPAGPAGPVGPVGARGPAGPQGPRGDKGETGEQGDRGIKGHRGFSGLQGPPGPPGSPGEQGPSGASGPAGPRGPPGSAGAPGKDGLNGLPGPIGPPGPRGRTGDAGPVGPPGPPGPPGPPGPPSAGFDFSFLPQPPQEKAHDGGRYYRAHHHHHH

SEQ ID NO: 8 - DNA, 3216 bp, Artificial Sequence
  source 1..3216: mol_type = other DNA; note = DNA sequence of gene COL1A1M1 encoding a1 (I) M1 with N-terminal Strep-Tag II tag and C-terminal 6 x His Tag
tggtctcatccacaatttgaaaagcaacttagttatggatacgatgaaaaatccacaggtggaatcagtgttcctggacctatgggtccatcaggtccaagaggtttaccaggacctccaggtgccccaggtccccagggatttcaaggtccaccaggagagcctggtgagccaggagcttctggtccacctggtccccctggaccacctggtcctccaggaaagaatggagatgatggtgaagctggaaaacctggaagacctggagaaagaggaccaccaggaccccagggtgccagaggactgccaggtaccgcaggtctgcctggaatgaaaggtcatagaggattttcaggattagacggtgcaaagggagacgctggacctgcaggaccaaagggtgagccaggaagtccaggagagaatggtgcaccaggacagccaggtccacctggactgcccggtgaaagaggtagacccggagcaccaggaccagcaggtgcaagaggaaatgatggagctacaggtgctgcaggacccccaggtccaacaggaccagccggtcctcccggtttcccaggtgccgttggagcaaaaggtgaagctggtccacagggtccaagaggttctgaaggtccacagggagttagaggagaaccaggaccccctggaccagctggtgcagcaggaccagctggtaaccctggtgctgacggtcagccaggtgctaagggagcaaatggagcaccaggaatagctggtgccccaggatttcccggtgctagaggtccaagtggtccacaaggaccaggaggtccacccggtcccaaaggaaacagtggagaaccaggtgcacccggttcaaagggagatacaggagctaaaggagagcccggtccagtgggtgttcagggaccacccggacctgctggagaggaaggtaaaagaggtgcaagaggtgagccaggaccaacaggtctgcctggtccccctggtgaaagaggtggtccaggtagtagaggatttccaggagctgatggtgttgcaggaccaaagggacccgcaggtgagagaggatcacccggtccagccggaccaaaaggatcaccaggagaagctggtagaccaggagaagctggtctgccaggtgctaaaggattgacaggatcacccggttcacctggtcctgatggaaagacaggacctccaggtcccgctggtcaggacggtagaccaggacccccaggacccccaggtgcaagaggtcaggcaggtgtaatgggtttccccggacctaaaggagcagctggagaacctggtaaagctggagagagaggagtgcctggaccccctggagctgttggtccagcaggaaaggatggtgaggcaggtgcacaaggtccacctggacccgctggacctgcaggtgagagaggagagcaaggtcccgcaggttctccaggttttcagggtttgccaggtccagccggtcctcctggagaggcaggaaagccaggagaacaaggagttccaggagacctgggtgcaccaggaccctctggtgcaagaggagagagaggatttcctggagaaagaggtgtgcagggaccaccaggtcccgccggtccaagaggagcaaatggagcccctggaaatgacggagctaagggtgacgctggtgcaccaggagcaccaggttctcaaggtgctcccggattgcagggtatgcctggagagagaggtgcagctggactgccaggtccaaaaggtgacagaggagacgccggtcctaagggagctgacggttctcctggaaaggacggtgtgagaggtttgacaggaccaataggtccacccggtcctgctggagcccctggagacaaaggtgaatcaggtccttccggtccagccggaccaacaggagcaagaggagcacctggagacagaggagagccaggtcctccaggacctgcaggtttcgctggtcctcccggagcagatggacagccaggagctaagggagaacccggtgacgctggtgctaagggagatgcaggtccaccaggtcctgctggtcctgctggacctcccggaccaataggtaatgttggagcacccggagcaaaaggtgccagaggttccgcaggtcctcccggagcaactggttttccaggagctgccggaagagtgggtccacctggtccttctggaaatgcaggaccaccaggtcctcctggtccagccggaaaggaaggtggaaagggacctagaggagaaacaggtcccgcaggtagacccggtgaggtgggtccacctggtccacccggtccagctggtgagaaaggaagtcctggagcagacggaccagctggtgcccctggtacaccaggaccccaaggaatagctggtcaaagaggtgttgttggtttaccaggtcagagaggagaaagaggttttccaggattaccaggtccctcaggtgagcccggaaaacagggtccctcaggagcaagtggtgaaagaggaccaccaggaccaatgggacctccaggattagctggtccaccaggagaatcaggaagagagggtgctcctggagcagaaggttcaccaggaagagacggttcacccggagccaagggagacagaggtgaaacaggtcccgcaggtccaccaggagcacccggagcccctggtgctccaggacctgtcggaccagcaggaaaatccggtgacagaggtgagactggacccgcaggtcctgctggtcctgttggaccagtgggtgcaagaggaccagcaggtccacaaggtccaagaggtgacaaaggtgagacaggtgagcagggtgacagaggaattaaaggtcacagaggattttcaggactgcagggaccacccggtcctcccggttccccaggagagcaaggtccatccggtgcatccggtccagctggacccagaggaccacctggttctgctggtgcaccaggtaaagatggattgaacggtttgcctggtccaataggacctcctggtccaagaggaagaactggtgacgccggtcccgtcggaccacccggtccaccaggtcccccaggtccacccggaccaccatccgcaggatttgatttctcattccttcctcaacctcctcaagagaaagcacatgatggaggtagatactatagagcccatcaccaccatcatcattaa

SEQ ID NO: 9 - protein, 1076 aa, Artificial Sequence
  source 1..1076: note = Amino acid sequence of a1 (II) M6 with N-terminal Strep-Tag II tag and C-terminal 6 x His Tag
EFWSHPQFEKQMAGGFDEKAGGAQLGPPQGPPGPPGPPGPPGPAGAPGPQGFQGNPGEPGEPGVSGPPGPPGPPGPPGKPGDDGEAGKPGKAGERGPPGPQGARGFPGTPGLPGVKGHRGYPGLDGAKGEAGAPGVKGESGSPGENGSPGPPGPPGLPGERGRTGPAGAAGARGNDGQPGPAGPPGPVGPAGGPGFPGAPGAKGEAGPTGARGPEGAQGPRGEPGTPGSPGPAGASGNPGTDGIPGAKGSAGAPGIAGAPGFPGPRGPPGPQGATGPLGPKGQTGEPGIAGFKGEQGPKGEPGPAGPQGAPGPAGEEGKRGARGEPGGVGPIGPPGERGAPGNRGFPGQDGLAGPKGAPGERGPSGLAGPKGANGDPGRPGEPGLPGARGLTGRPGDAGPQGKVGPSGAPGEDGRPGPPGPQGARGQPGVMGFPGPKGANGEPGKAGEKGLPGAPGLRGLPGKDGETGAAGPPGPAGPAGERGEQGAPGPSGFQGLPGPPGPPGEGGKPGDQGVPGEAGAPGLVGPRGERGFPGERGSPGAQGLQGPRGLPGTPGTDGPKGASGPAGPPGAQGPPGLQGMPGERGAAGIAGPKGDRGDVGEKGPEGAPGKDGGRGLTGPIGPPGPAGANGEKGEVGPPGPAGSAGARGAPGERGETGPPGPAGFAGPPGADGQPGAKGEQGEAGQKGDAGAPGPQGPSGAPGPQGPTGVTGPKGARGAQGPPGATGFPGAAGRVGPPGSNGNPGPPGPPGPSGKDGPKGARGDSGPPGRAGEPGLQGPAGPPGEKGEPGDDGPSGAEGPPGPQGLAGQRGIVGLPGQRGERGFPGLPGPSGEPGKQGAPGASGDRGPPGPVGPPGLTGPAGEPGREGSPGADGPPGRDGAAGVKGDRGETGAVGAPGAPGPPGSPGPAGPTGKQGDRGEAGAQGPMGPSGPAGARGIQGPQGPRGDKGEAGEPGERGLKGHRGFTGLQGLPGPPGPSGDQGASGPAGPSGPRGPPGPVGPSGKDGANGIPGPIGPPGPRGRSGETGPAGPPGNPGPPGPPGPPGPGIDMSAFAGLGPREKGPDPLQYMRAHHHHHH

SEQ ID NO: 10 - DNA, 3231 bp, Artificial Sequence
  source 1..3231: mol_type = other DNA; note = DNA sequence of gene COL2A1M6 encoding a1 (II) M6 with N-terminal Strep-Tag II tag and C-terminal 6 x His Tag
gaattctggagtcatcctcaattcgaaaaacaaatggctggtggattcgatgaaaaggctggtggagcccaattaggtcctccacaaggtcctcccggtccacctggtcctcccggtcctccaggtcccgccggtgctcctggaccacagggtttccaaggaaaccccggtgaaccaggtgagcctggtgtttcaggtcctcccggtcctccaggaccacctggaccaccaggaaagcctggtgacgacggagaagctggtaaaccaggaaaggcaggagagagaggtccacctggacctcagggtgccagaggtttcccaggtacccctggtcttcctggtgtcaagggtcatagaggttaccccggtttggatggtgccaagggtgaagccggtgcccctggtgttaagggtgaatcaggaagtcccggtgaaaatggaagtcccggtccacccggtccacctggactgccaggtgagagaggaagaaccggaccagctggtgctgcaggtgctagaggaaatgacggacagcccggaccagccggacctcccggtcctgttgggcccgcaggtggtcctggtttccctggtgctcctggagccaaaggagaagccggacccaccggagccagaggtcccgagggagcacagggacctagaggagaaccaggtacaccaggtagtcccggtcctgctggtgcatcaggaaatcccggaactgacggtattccaggagcaaagggatctgcaggagcaccaggaatagctggtgctcctggatttccaggtcccagaggacctcccggtcctcaaggagcaacaggtcctttgggaccaaaaggtcaaacaggagaaccaggtattgctggattcaaaggagagcaaggtccaaagggagagcccggtcccgcaggtccccaaggagccccaggaccagctggtgaagaaggaaaaagaggagccagaggtgaacctggaggagtaggacctattggtcctcctggtgagagaggtgctcccggaaacagaggttttcctggtcaagatggtctggctggacctaaaggtgctccaggagagagaggaccttcaggacttgctggtccaaaaggtgctaacggagatccaggaagacccggtgaacctggtctgcctggagctagaggattaacaggaagaccaggtgacgcaggtccccagggtaaagtgggtcccagtggtgccccaggtgaagatggaagacctggtcctcccggaccccaaggtgcaagaggtcagcctggagtgatgggatttcctggacccaagggtgctaacggagaacctggaaaagctggtgagaaaggactgcccggtgccccaggtcttagaggtttgccaggtaaagatggagaaacaggagccgcaggaccacccggtccagccggaccagcaggagagagaggtgaacaaggagcacctggtccaagtggttttcagggtcttccaggtccccctggtccaccaggagagggaggtaaaccaggtgaccaaggtgtccctggagaagcaggtgcacccggtcttgtgggtccaagaggtgaaagaggattccctggtgagagaggatctcccggagcccagggacttcaaggtcctagaggtctgccaggtacccctggtacagacggaccaaagggagcatcaggacccgctggacctcccggagcccaaggtcctccaggtttacaaggtatgcctggtgaaagaggtgctgcaggtatagctggaccaaaaggagacagaggtgacgttggtgagaagggtcccgaaggagcccctggaaaagatggtggaagaggattaacaggtcctataggaccacccggtccagccggtgctaatggagaaaaaggagaagtaggtcctccaggtccagcaggatctgcaggtgctagaggtgcccctggagagagaggtgaaacaggaccacctggtccagctggtttcgctggtcccccaggagctgatggacagcccggtgcaaaaggtgaacaaggagaagccggacagaagggagatgctggagcccccggtccacaaggtccctcaggagcaccaggtcctcaaggtccaactggtgtgaccgggccaaagggtgcaagaggagcacagggacctccaggagcaacaggtttcccaggagctgctggtagagtcggtccacccggatctaatggtaaccccggaccaccaggaccacctggaccatctggaaaggatggacccaaaggagcaagaggagattcaggaccacccggaagagcaggagaacctggattacagggtcccgccggtccaccaggagagaaaggagagcccggagatgatggtccctcaggtgcagagggacccccaggaccccaaggtctggcaggtcaaagaggtatagtgggtcttccaggtcaaagaggtgaaagaggatttccaggacttccaggtccttcaggtgaacccggtaaacagggagcccccggagcctcaggtgacagaggtcctccaggaccagtaggacccccaggtttaaccggaccagcaggtgagccaggaagagaaggttctcctggagccgatggacctccaggaagagacggtgcagctggtgttaagggtgacagaggtgaaactggagccgtaggagccccaggtgcccccggaccacccggatcacccggacctgcaggtcctactggtaaacaaggagatagaggagaagccggtgcccagggtcctatgggtccttctggtcctgcaggagcaagaggtatacaaggtccacagggtcccagaggtgacaagggtgaagcaggagaacccggtgagagaggtctgaagggtcatagaggattcaccgggttacagggtttgccaggaccccctggaccaagtggtgaccagggtgcatccggtccagcaggtccttctggaccaagaggtcctcccggtccagttggtccatcaggtaaagacggagccaacggtatcccaggtcccatcggtcctccaggtcctagaggaagaagtggagagactggtcctgctggacctcctggaaaccctggtcctccaggacctccaggtcctccaggtcccggaatagatatgtccgctttcgctggattgggaccaagagagaaaggtcctgaccctcttcaatatatgagagcacaccatcaccatcatcactaa